European Patent Specification EP 4 058 593 B1, published July 29, 2026. Title: METHODS OF DETECTING A FUSION GENE ENCODING A NEOANTIGEN. Applicant: FOUNDATION MEDICINE, INC. Application Not Yet Assigned. The sequence listing filed with the application follows.

SEQUENCE LISTING (40 sequences)

SEQ ID NO: 1 - protein, 9 aa, Artificial Sequence
  Synthetic Construct
SSYGQQSEK

SEQ ID NO: 2 - protein, 9 aa, Artificial Sequence
  Synthetic Construct
YGQQSEKPY

SEQ ID NO: 3 - protein, 16 aa, Artificial Sequence
  Synthetic Construct
SSSYGQQSEKPYQCDF

SEQ ID NO: 4 - protein, 362 aa, Artificial Sequence
  Synthetic Construct
MASTDYSTYSQAAAQQGYSAYTAQPTQGYAQTTQAYGQQSYGTYGQPTDVSYTQAQTTATYGQTAYATSYGQPPTGYTTPTAPQAYSQPVQGYGTGAYDTTTATVTTTQASYAAQSAYGTQPAYPAYGQQPAATAPTRPQDGNKPTETSQPQSSTGGYNQPSLGYGQSNYSYPQVPGSYPMQPVTAPPSYPPTSYSSTQPTSYDQSSYSQQNTYGQPSSYGQQSSYGQQSSYGQQPPTSYPPQTGSYSQAPSQYSQQSSSYGQQSEKPYQCDFKDCERRFSRSDQLKRHQRRHTGVKPFQCKTCQRKFSRSDHLKTHTRTHTGEKPFSCRWPSCQKKFARSDELVRHHNMHQRNMTKLQLAL

SEQ ID NO: 5 - protein, 365 aa, Artificial Sequence
  Synthetic Construct
MASTDYSTYSQAAAQQGYSAYTAQPTQGYAQTTQAYGQQSYGTYGQPTDVSYTQAQTTATYGQTAYATSYGQPPTGYTTPTAPQAYSQPVQGYGTGAYDTTTATVTTTQASYAAQSAYGTQPAYPAYGQQPAATAPTRPQDGNKPTETSQPQSSTGGYNQPSLGYGQSNYSYPQVPGSYPMQPVTAPPSYPPTSYSSTQPTSYDQSSYSQQNTYGQPSSYGQQSSYGQQSSYGQQPPTSYPPQTGSYSQAPSQYSQQSSSYGQQSEKPYQCDFKDCERRFSRSDQLKRHQRRHTGVKPFQCKTCQRKFSRSDHLKTHTRTHTGKTSEKPFSCRWPSCQKKFARSDELVRHHNMHQRNMTKLQLAL

SEQ ID NO: 6 - protein, 306 aa, Artificial Sequence
  Synthetic Construct
MASTDYSTYSQAAAQQGYSAYTAQPTQGYAQTTQAYGQQSYGTYGQPTDVSYTQAQTTATYGQTAYATSYGQPPTGYTTPTAPQAYSQPVQGYGTGAYDTTTATVTTTQASYAAQSAYGTQPAYPAYGQQPAATAPTSYSSTQPTSYDQSSYSQQNTYGQPSSYGQQSSYGQQSSYGQQPPTSYPPQTGSYSQAPSQYSQQSSSYGQQSEKPYQCDFKDCERRFSRSDQLKRHQRRHTGVKPFQCKTCQRKFSRSDHLKTHTRTHTGEKPFSCRWPSCQKKFARSDELVRHHNMHQRNMTKLQLAL

SEQ ID NO: 7 - protein, 368 aa, Artificial Sequence
  Synthetic Construct
MASTDYSTYSQAAAQQGYSAYTAQPTQGYAQTTQAYGQQSYGTYGQPTDVSYTQAQTTATYGQTAYATSYGQPPTVEGTSTGYTTPTAPQAYSQPVQGYGTGAYDTTTATVTTTQASYAAQSAYGTQPAYPAYGQQPAATAPTRPQDGNKPTETSQPQSSTGGYNQPSLGYGQSNYSYPQVPGSYPMQPVTAPPSYPPTSYSSTQPTSYDQSSYSQQNTYGQPSSYGQQSSYGQQSSYGQQPPTSYPPQTGSYSQAPSQYSQQSSSYGQQSEKPYQCDFKDCERRFSRSDQLKRHQRRHTGVKPFQCKTCQRKFSRSDHLKTHTRTHTGEKPFSCRWPSCQKKFARSDELVRHHNMHQRNMTKLQLAL

SEQ ID NO: 8 - protein, 362 aa, Artificial Sequence; identical to SEQ ID NO: 4
  Synthetic Construct

SEQ ID NO: 9 - protein, 309 aa, Artificial Sequence
  Synthetic Construct
MASTDYSTYSQAAAQQGYSAYTAQPTQGYAQTTQAYGQQSYGTYGQPTDVSYTQAQTTATYGQTAYATSYGQPPTGYTTPTAPQAYSQPVQGYGTGAYDTTTATVTTTQASYAAQSAYGTQPAYPAYGQQPAATAPTSYSSTQPTSYDQSSYSQQNTYGQPSSYGQQSSYGQQSSYGQQPPTSYPPQTGSYSQAPSQYSQQSSSYGQQSEKPYQCDFKDCERRFSRSDQLKRHQRRHTGVKPFQCKTCQRKFSRSDHLKTHTRTHTGKTSEKPFSCRWPSCQKKFARSDELVRHHNMHQRNMTKLQLAL

SEQ ID NO: 10 - protein, 371 aa, Artificial Sequence
  Synthetic Construct
MASTDYSTYSQAAAQQGYSAYTAQPTQGYAQTTQAYGQQSYGTYGQPTDVSYTQAQTTATYGQTAYATSYGQPPTVEGTSTGYTTPTAPQAYSQPVQGYGTGAYDTTTATVTTTQASYAAQSAYGTQPAYPAYGQQPAATAPTRPQDGNKPTETSQPQSSTGGYNQPSLGYGQSNYSYPQVPGSYPMQPVTAPPSYPPTSYSSTQPTSYDQSSYSQQNTYGQPSSYGQQSSYGQQSSYGQQPPTSYPPQTGSYSQAPSQYSQQSSSYGQQSEKPYQCDFKDCERRFSRSDQLKRHQRRHTGVKPFQCKTCQRKFSRSDHLKTHTRTHTGKTSEKPFSCRWPSCQKKFARSDELVRHHNMHQRNMTKLQLAL

SEQ ID NO: 11 - protein, 365 aa, Artificial Sequence; identical to SEQ ID NO: 5
  Synthetic Construct

SEQ ID NO: 12 - protein, 439 aa, Artificial Sequence
  Synthetic Construct
QVQLVESGGGVVQPGRSLRLDCKASGITFSNSGMHWVRQAPGKGLEWVAVIWYDGSKRYYADSVKGRFTISRDNSKNTLFLQMNSLRAEDTAVYYCATNDDYWGQGTLVTVSSASTKGPSVFPLAPCSRSTSESTAALGCLVKDYFPEPVTVSWNSGALTSGVHTFPAVLQSSGLYSLSSVVTVPSSSLGTKTYTCNVDHKPSNTKVDKRVESKYGPPCPPCPAPEFLGGPSVFLFPPKPKDTLMISRTPEVTCVVVDVSQEDPEVQFNWYVDGVEVHNAKTKPREEQFNSTYRVVSVLTVLHQDWLNGKEYKCKVSNKGLPSSIEKTISKAKGQPREPQVYTLPPSQEEMTKNQVSLTCLVKGFYPSDIAVEWESNGQPENNYKTTPPVLDSDGSFFLYSRLTVDKSRWQEGNVFSCSVMHEALHNHYTQKSLSLSLG

SEQ ID NO: 13 - protein, 214 aa, Artificial Sequence
  Synthetic Construct
EIVLTQSPATLSLSPGERATLSCRASQSVSSYLAWYQQKPGQAPRLLIYDASNRATGIPARFSGSGSGTDFTLTISSLEPEDFAVYYCQQSSNWPRTFGQGTKVEIKRTVAAPSVFIFPPSDEQLKSGTASVVCLLNNFYPREAKVQWKVDNALQSGNSQESVTEQDSKDSTYSLSSTLTLSKADYEKHKVYACEVTHQGLSSPVTKSFNRGEC

SEQ ID NO: 14 - protein, 446 aa, Artificial Sequence
  Synthetic Construct
QVQLVQSGVEVKKPGASVKVSCKASGYTFTNYYMYWVRQAPGQGLEWMGGINPSNGGTNFNEKFKNRVTLTTDSSTTTAYMELKSLQFDDTAVYYCARRDYRFDMGFDYWGQGTTVTVSSASTKGPSVFPLAPCSRSTSESTAALGCLVKDYFPEPVTVSWNSGALTSGVHTFPAVLQSSGLYSLSSVVTVPSSSLGTKTYTCNVDHKPSNTKVDKRVESKYGPPCPPCPAPEFLGGPSVFLFPPKPKDTLMISRTPEVTCVVVDVSQEDPEVQFNWYVDGVEVHNAKTKPREEQFNSTYRVVSVLTVLHQDWLNGKEYKCKVSNKGLPSSIEKTISKAKGQPREPQVYTLPPSQEEMTKNQVSLTCLVKGFYPSDIAVEWESNGQPENNYKTTPPVLDSDGSFFLYSRLTVDKSRWQEGNVFSCSVMHEALHNHYTQKSLSLSLG

SEQ ID NO: 15 - protein, 218 aa, Artificial Sequence
  Synthetic Construct
EIVLTQSPATLSLSPGERATLSCRASKGVSTSGYSYLHWYQQKPGQAPRLLIYLASYLESGVPARFSGSGSGTDFTLTISSLEPEDFAVYYCQHSRDLPLTFGGGTKVEIKRTVAAPSVFIFPPSDEQLKSGTASVVCLLNNFYPREAKVQWKVDNALQSGNSQESVTEQDSKDSTYSLSSTLTLSKADYEKHKVYACEVTHQGLSSPVTKSFNRGEC

SEQ ID NO: 16 - protein, 10 aa, Artificial Sequence
  Synthetic Construct
GFTFSDSWIH

SEQ ID NO: 17 - protein, 18 aa, Artificial Sequence
  Synthetic Construct
AWISPYGGSTYYADSVKG

SEQ ID NO: 18 - protein, 9 aa, Artificial Sequence
  Synthetic Construct
RHWPGGFDY

SEQ ID NO: 19 - protein, 11 aa, Artificial Sequence
  Synthetic Construct
RASQDVSTAVA

SEQ ID NO: 20 - protein, 7 aa, Artificial Sequence
  Synthetic Construct
SASFLYS

SEQ ID NO: 21 - protein, 9 aa, Artificial Sequence
  Synthetic Construct
QQYLYHPAT

SEQ ID NO: 22 - protein, 118 aa, Artificial Sequence [sequence omitted]

SEQ ID NO: 23 - protein, 108 aa, Artificial Sequence
  Synthetic Construct
DIQMTQSPSSLSASVGDRVTITCRASQDVSTAVAWYQQKPGKAPKLLIYSASFLYSGVPSRFSGSGSGTDFTLTISSLQPEDFATYYCQQYLYHPATFGQGTKVEIKR

SEQ ID NO: 24 - protein, 447 aa, Artificial Sequence
  Synthetic Construct
EVQLVESGGGLVQPGGSLRLSCAASGFTFSDSWIHWVRQAPGKGLEWVAWISPYGGSTYYADSVKGRFTISADTSKNTAYLQMNSLRAEDTAVYYCARRHWPGGFDYWGQGTLVTVSSASTKGPSVFPLAPSSKSTSGGTAALGCLVKDYFPEPVTVSWNSGALTSGVHTFPAVLQSSGLYSLSSVVTVPSSSLGTQTYICNVNHKPSNTKVDKKVEPKSCDKTHTCPPCPAPELLGGPSVFLFPPKPKDTLMISRTPEVTCVVVDVSHEDPEVKFNWYVDGVEVHNAKTKPREEQYASTYRVVSVLTVLHQDWLNGKEYKCKVSNKALPAPIEKTISKAKGQPREPQVYTLPPSREEMTKNQVSLTCLVKGFYPSDIAVEWESNGQPENNYKTTPPVLDSDGSFFLYSKLTVDKSRWQQGNVFSCSVMHEALHNHYTQKSLSLSPG

SEQ ID NO: 25 - protein, 214 aa, Artificial Sequence
  Synthetic Construct
DIQMTQSPSSLSASVGDRVTITCRASQDVSTAVAWYQQKPGKAPKLLIYSASFLYSGVPSRFSGSGSGTDFTLTISSLQPEDFATYYCQQYLYHPATFGQGTKVEIKRTVAAPSVFIFPPSDEQLKSGTASVVCLLNNFYPREAKVQWKVDNALQSGNSQESVTEQDSKDSTYSLSSTLTLSKADYEKHKVYACEVTHQGLSSPVTKSFNRGEC

SEQ ID NO: 26 - protein, 449 aa, Artificial Sequence
  Synthetic Construct
EVQLLESGGGLVQPGGSLRLSCAASGFTFSSYIMMWVRQAPGKGLEWVSSIYPSGGITFYADTVKGRFTISRDNSKNTLYLQMNSLRAEDTAVYYCARIKLGTVTTVDYWGQGTLVTVSSASTKGPSVFPLAPSSKSTSGGTAALGCLVKDYFPEPVTVSWNSGALTSGVHTFPAVLQSSGLYSLSSVVTVPSSSLGTQTYICNVNHKPSNTKVDKKVEPKSCDKTHTCPPCPAPELLGGPSVFLFPPKPKDTLMISRTPEVTCVVVDVSHEDPEVKFNWYVDGVEVHNAKTKPREEQYNSTYRVVSVLTVLHQDWLNGKEYKCKVSNKALPAPIEKTISKAKGQPREPQVYTLPPSRDELTKNQVSLTCLVKGFYPSDIAVEWESNGQPENNYKTTPPVLDSDGSFFLYSKLTVDKSRWQQGNVFSCSVMHEALHNHYTQKSLSLSPG

SEQ ID NO: 27 - protein, 216 aa, Artificial Sequence
  Synthetic Construct
QSALTQPASVSGSPGQSITISCTGTSSDVGGYNYVSWYQQHPGKAPKLMIYDVSNRPSGVSNRFSGSKSGNTASLTISGLQAEDEADYYCSSYTSSSTRVFGTGTKVTVLGQPKANPTVTLFPPSSEELQANKATLVCLISDFYPGAVTVAWKADGSPVKAGVETTKPSKQSNNKYAASSYLSLTPEQWKSHRSYSCQVTHEGSTVEKTVAPTECS

SEQ ID NO: 28 - protein, 450 aa, Artificial Sequence
  Synthetic Construct
EVQLVESGGGLVQPGGSLRLSCAASGFTFSRYWMSWVRQAPGKGLEWVANIKQDGSEKYYVDSVKGRFTISRDNAKNSLYLQMNSLRAEDTAVYYCAREGGWFGELAFDYWGQGTLVTVSSASTKGPSVFPLAPSSKSTSGGTAALGCLVKDYFPEPVTVSWNSGALTSGVHTFPAVLQSSGLYSLSSVVTVPSSSLGTQTYICNVNHKPSNTKVDKRVEPKSCDKTHTCPPCPAPEFEGGPSVFLFPPKPKDTLMISRTPEVTCVVVDVSHEDPEVKFNWYVDGVEVHNAKTKPREEQYNSTYRVVSVLTVLHQDWLNGKEYKCKVSNKALPASIEKTISKAKGQPREPQVYTLPPSREEMTKNQVSLTCLVKGFYPSDIAVEWESNGQPENNYKTTPPVLDSDGSFFLYSKLTVDKSRWQQGNVFSCSVMHEALHNHYTQKSLSLSPG

SEQ ID NO: 29 - protein, 215 aa, Artificial Sequence
  Synthetic Construct
EIVLTQSPGTLSLSPGERATLSCRASQRVSSSYLAWYQQKPGQAPRLLIYDASSRATGIPDRFSGSGSGTDFTLTISRLEPEDFAVYYCQQYGSLPWTFGQGTKVEIKRTVAAPSVFIFPPSDEQLKSGTASVVCLLNNFYPREAKVQWKVDNALQSGNSQESVTEQDSKDSTYSLSSTLTLSKADYEKHKVYACEVTHQGLSSPVTKSFNRGEC

SEQ ID NO: 30 - protein, 118 aa, Artificial Sequence
  Synthetic Construct
QVQLVESGGGVVQPGRSLRLSCAASGFTFSSYTMHWVRQAPGKGLEWVTFISYDGNNKYYADSVKGRFTISRDNSKNTLYLQMNSLRAEDTAIYYCARTGWLGPFDYWGQGTLVTVSS

SEQ ID NO: 31 - protein, 108 aa, Artificial Sequence
  Synthetic Construct
EIVLTQSPGTLSLSPGERATLSCRASQSVGSSYLAWYQQKPGQAPRLLIYGAFSRATGIPDRFSGSGSGTDFTLTISRLEPEDFAVYYCQQYGSSPWTFGQGTKVEIK

SEQ ID NO: 32 - protein, 16 aa, Artificial Sequence
  Synthetic Construct
SSSYGQQSEKPYQCDF

SEQ ID NO: 33 - protein, 9 aa, Artificial Sequence
  Synthetic Construct
SSSYGQQSE

SEQ ID NO: 34 - protein, 9 aa, Artificial Sequence
  Synthetic Construct
SSYGQQSEK

SEQ ID NO: 35 - protein, 9 aa, Artificial Sequence
  Synthetic Construct
SYGQQSEKP

SEQ ID NO: 36 - protein, 9 aa, Artificial Sequence
  Synthetic Construct
YGQQSEKPY

SEQ ID NO: 37 - protein, 9 aa, Artificial Sequence
  Synthetic Construct
GQQSEKPYQ

SEQ ID NO: 38 - protein, 9 aa, Artificial Sequence
  Synthetic Construct
QQSEKPYQC

SEQ ID NO: 39 - protein, 9 aa, Artificial Sequence
  Synthetic Construct
QSEKPYQCD

SEQ ID NO: 40 - protein, 9 aa, Artificial Sequence
  Synthetic Construct
SEKPYQCDF